European Patent Specification EP 4 132 943 B1, published May 29, 2024. Title: IMMUNOGLOBULIN BINDING PROTEINS FOR AFFINITY PURIFICATION. Applicant: Navigo Proteins GmbH. The sequence listing filed with the application follows.

SEQUENCE LISTING (60 sequences)

SEQ ID NO: 1 - protein, 58 aa, Artificial Sequence
  cs26 (CID186352)
IAAQHDKDQQAAFYEILHLPNLTEEQRNAFIQSLRDDPSVSLEILAEAKKLNDAQAPK

SEQ ID NO: 2 - protein, 58 aa, Artificial Sequence
  cs26 46C
IAAQHDKDQQAAFYEILHLPNLTEEQRNAFIQSLRDDPSVSLEILCEAKKLNDAQAPK

SEQ ID NO: 3 - protein, 58 aa, Artificial Sequence
  cs26 43C (CID203447)
IAAQHDKDQQAAFYEILHLPNLTEEQRNAFIQSLRDDPSVSLCILAEAKKLNDAQAPK

SEQ ID NO: 4 - protein, 58 aa, Artificial Sequence
  cs26 D8I
IAAQHDKIQQAAFYEILHLPNLTEEQRNAFIQSLRDDPSVSLEILAEAKKLNDAQAPK

SEQ ID NO: 5 - protein, 58 aa, Artificial Sequence
  cs26 8I 43C (CID203550)
IAAQHDKIQQAAFYEILHLPNLTEEQRNAFIQSLRDDPSVSLCILAEAKKLNDAQAPK

SEQ ID NO: 6 - protein, 58 aa, Artificial Sequence
  cs26 8F
IAAQHDKFQQAAFYEILHLPNLTEEQRNAFIQSLRDDPSVSLEILAEAKKLNDAQAPK

SEQ ID NO: 7 - protein, 58 aa, Artificial Sequence
  cs26 8Y (CID203532)
IAAQHDKYQQAAFYEILHLPNLTEEQRNAFIQSLRDDPSVSLEILAEAKKLNDAQAPK

SEQ ID NO: 8 - protein, 58 aa, Artificial Sequence
  cs26 8W
IAAQHDKWQQAAFYEILHLPNLTEEQRNAFIQSLRDDPSVSLEILAEAKKLNDAQAPK

SEQ ID NO: 9 - protein, 58 aa, Artificial Sequence
  cs26 8L
IAAQHDKLQQAAFYEILHLPNLTEEQRNAFIQSLRDDPSVSLEILAEAKKLNDAQAPK

SEQ ID NO: 10 - protein, 58 aa, Artificial Sequence
  cs26 6I (CID203522)
IAAQHIKDQQAAFYEILHLPNLTEEQRNAFIQSLRDDPSVSLEILAEAKKLNDAQAPK

SEQ ID NO: 11 - protein, 58 aa, Artificial Sequence
  cs26 6Y (203531)
IAAQHYKDQQAAFYEILHLPNLTEEQRNAFIQSLRDDPSVSLEILAEAKKLNDAQAPK

SEQ ID NO: 12 - protein, 58 aa, Artificial Sequence
  cs26 6W
IAAQHWKDQQAAFYEILHLPNLTEEQRNAFIQSLRDDPSVSLEILAEAKKLNDAQAPK

SEQ ID NO: 13 - protein, 58 aa, Artificial Sequence
  cs26 6L
IAAQHLKDQQAAFYEILHLPNLTEEQRNAFIQSLRDDPSVSLEILAEAKKLNDAQAPK

SEQ ID NO: 14 - protein, 58 aa, Artificial Sequence
  cs26 6L 43C (203524)
IAAQHLKDQQAAFYEILHLPNLTEEQRNAFIQSLRDDPSVSCEILAEAKKLNDAQAPK

SEQ ID NO: 15 - protein, 58 aa, Artificial Sequence
  cs26 4I
IAAIHDKDQQAAFYEILHLPNLTEEQRNAFIQSLRDDPSVSLEILAEAKKLNDAQAPK

SEQ ID NO: 16 - protein, 58 aa, Artificial Sequence
  cs26 4F (203494)
IAAFHDKDQQAAFYEILHLPNLTEEQRNAFIQSLRDDPSVSLEILAEAKKLNDAQAPK

SEQ ID NO: 17 - protein, 58 aa, Artificial Sequence
  cs26 4W (203502)
IAAWHDKDQQAAFYEILHLPNLTEEQRNAFIQSLRDDPSVSLEILAEAKKLNDAQAPK

SEQ ID NO: 18 - protein, 58 aa, Artificial Sequence
  cs26 4L
IAALHDKDQQAAFYEILHLPNLTEEQRNAFIQSLRDDPSVSLEILAEAKKLNDAQAPK

SEQ ID NO: 19 - protein, 58 aa, Artificial Sequence
  cs26 4Y
IAAYHDKDQQAAFYEILHLPNLTEEQRNAFIQSLRDDPSVSLEILAEAKKLNDAQAPK

SEQ ID NO: 20 - protein, 58 aa, Artificial Sequence
  cs26 8I 14H
IAAQHDKIQQAAFHEILHLPNLTEEQRNAFIQSLRDDPSVSLEILAEAKKLNDAQAPK

SEQ ID NO: 21 - protein, 58 aa, Artificial Sequence
  cs26 8I 14H 46C
IAAQHDKIQQAAFHEILHLPNLTEEQRNAFIQSLRDDPSVSLEILCEAKKLNDAQAPK

SEQ ID NO: 22 - protein, 58 aa, Artificial Sequence
  cs26 8I 28H 46C
IAAQHDKIQQAAFYEILHLPNLTEEQRHAFIQSLRDDPSVSLEILCEAKKLNDAQAPK

SEQ ID NO: 23 - protein, 56 aa, Artificial Sequence
  cs26 8I 14H 43C  del1 del2
AQHDKIQQAAFHEILHLPNLTEEQRNAFIQSLRDDPSVSLCILAEAKKLNDAQAPK

SEQ ID NO: 24 - protein, 56 aa, Artificial Sequence
  cs26 8I 28H 43C del1 del2
AQHDKIQQAAFYEILHLPNLTEEQRHAFIQSLRDDPSVSLCILAEAKKLNDAQAPK

SEQ ID NO: 25 - protein, 58 aa, Artificial Sequence
  cs27 8I
IAAKFDEIQQAAFYEILHLPNLTEEQRNAFIQSLRDDPSVSLEVLGEAQKLNDSQAPK

SEQ ID NO: 26 - protein, 58 aa, Artificial Sequence
  cs27 8I 14H
IAAKFDEIQQAAFHEILHLPNLTEEQRNAFIQSLRDDPSVSLEVLGEAQKLNDSQAPK

SEQ ID NO: 27 - protein, 58 aa, Artificial Sequence
  cs27 8I 28H
IAAKFDEIQQAAFYEILHLPNLTEEQRHAFIQSLRDDPSVSLEVLGEAQKLNDSQAPK

SEQ ID NO: 28 - protein, 58 aa, Artificial Sequence
  cs59 8I
IDAKFDEIQQAAFYEILHLPNLTEDQRNAFIQSLRDDPSVSLALLAEAKKLNDAQAPP

SEQ ID NO: 29 - protein, 58 aa, Artificial Sequence
  cs59 8I 14H
IDAKFDEIQQAAFHEILHLPNLTEDQRNAFIQSLRDDPSVSLALLAEAKKLNDAQAPP

SEQ ID NO: 30 - protein, 58 aa, Artificial Sequence
  cs59 8I 28H
IDAKFDEIQQAAFYEILHLPNLTEDQRHAFIQSLRDDPSVSLALLAEAKKLNDAQAPP

SEQ ID NO: 31 - protein, 58 aa, Artificial Sequence
  cs60 8I
IDAKFDEIAQAAFYEILHLPNLTEDQRNAFIQSLRDDPSVSLALLAEAKKLNDAQAPP

SEQ ID NO: 32 - protein, 58 aa, Artificial Sequence
  cs60 8I 14H
IDAKFDEIAQAAFHEILHLPNLTEDQRNAFIQSLRDDPSVSLALLAEAKKLNDAQAPP

SEQ ID NO: 33 - protein, 58 aa, Artificial Sequence
  cs60 8I 28H
IDAKFDEIAQAAFYEILHLPNLTEDQRHAFIQSLRDDPSVSLALLAEAKKLNDAQAPP

SEQ ID NO: 34 - protein, 58 aa, Artificial Sequence
  cs14 8I
IAAKHDKIQQAAFYEILHLPNLTEDQRNAFIQSLRDDPSVSLEILGEAKKLNDAQAPP

SEQ ID NO: 35 - protein, 58 aa, Artificial Sequence
  cs14 8I 14H
IAAKHDKIQQAAFHEILHLPNLTEDQRNAFIQSLRDDPSVSLEILGEAKKLNDAQAPP

SEQ ID NO: 36 - protein, 58 aa, Artificial Sequence
  cs14 8I 28H
IAAKHDKIQQAAFYEILHLPNLTEDQRHAFIQSLRDDPSVSLEILGEAKKLNDAQAPP

SEQ ID NO: 37 - protein, 114 aa, Artificial Sequence
  dimer
AQHDKIQQAAFYEILHLPNLTEEQRNAFIQSLRDDPSVSLCILAEAKKLNDAQAPKIAAQHDKIQQAAFYEILHLPNLTEEQRNAFIQSLRDDPSVSLEILAEAKKLNDAQAPK

SEQ ID NO: 38 - protein, 58 aa, Artificial Sequence
  PAdelFc
IAAQHDKDQSAADSEILHLPNLTEEQRNAFRQSLSDDPSVSLEILAEAKKLNDAQAPK

SEQ ID NO: 39 - protein, 58 aa, Artificial Sequence
  PAdelFc
IAAQHDKIQQAADKEILHLPNLTEEQRNKFRQSLRDDPSVSAEILAEAKKLNDAQAPK

SEQ ID NO: 40 - protein, 56 aa, Artificial Sequence
  cs26 8I 14H 46C del2N
AQHDKIQQAAFHEILHLPNLTEEQRNAFIQSLRDDPSVSLEILCEAKKLNDAQAPK

SEQ ID NO: 41 - protein, 59 aa, Artificial Sequence
  cs26 8I 14H 29K c-term cys
IAAQHDKIQQAAFHEILHLPNLTEEQRNKFIQSLRDDPSVSLEILEEAKKLNDAQAPKC

SEQ ID NO: 42 - protein, 56 aa, Artificial Sequence
  cs26 8I 14H 29K del2N
AQHDKIQQAAFHEILHLPNLTEEQRNKFIQSLRDDPSVSLEILAEAKKLNDAQAPK

SEQ ID NO: 43 - protein, 58 aa, Artificial Sequence
  cs26 8I 14H 29K
IAAQHDKIQQAAFHEILHLPNLTEEQRNKFIQSLRDDPSVSLEILAEAKKLNDAQAPK

SEQ ID NO: 44 - protein, 47 aa, Artificial Sequence
  core of SEQ43
IQQAAFHEILHLPNLTEEQRNKFIQSLRDDPSVSLEILAEAKKLNDA

SEQ ID NO: 45 - protein, 58 aa, Artificial Sequence
  cs26 8I 14H 29K 43C
IAAQHDKIQQAAFHEILHLPNLTEEQRNKFIQSLRDDPSVSLCILAEAKKLNDAQAPK

SEQ ID NO: 46 - protein, 56 aa, Artificial Sequence
  cs26 8I 14H 29K 46C  del2N
AQHDKIQQAAFHEILHLPNLTEEQRNKFIQSLRDDPSVSLEILCEAKKLNDAQAPK

SEQ ID NO: 47 - protein, 58 aa, Artificial Sequence
  cs26 8I 14H 29K 46C
IAAQHDKIQQAAFHEILHLPNLTEEQRNKFIQSLRDDPSVSLEILCEAKKLNDAQAPK

SEQ ID NO: 48 - protein, 47 aa, Artificial Sequence
  core of SEQ ID NO: 47
IQQAAFHEILHLPNLTEEQRNKFIQSLRDDPSVSLEILCEAKKLNDA

SEQ ID NO: 49 - protein, 58 aa, Artificial Sequence
  cs26 8I 28H 29K 46C
IAAQHDKIQQAAFYEILHLPNLTEEQRHKFIQSLRDDPSVSLEILCEAKKLNDAQAPK

SEQ ID NO: 50 - protein, 116 aa, Artificial Sequence
  dimer of SEQ ID NO: 21 and SEQ ID NO: 20
IAAQHDKIQQAAFHEILHLPNLTEEQRNAFIQSLRDDPSVSLEILCEAKKLNDAQAPKIAAQHDKIQQAAFHEILHLPNLTEEQRNAFIQSLRDDPSVSLEILAEAKKLNDAQAPK

SEQ ID NO: 51 - protein, 114 aa, Artificial Sequence
  dimer of SEQ ID NO: 46 and SEQ ID NO: 43
AQHDKIQQAAFHEILHLPNLTEEQRNKFIQSLRDDPSVSLEILCEAKKLNDAQAPKIAAQHDKIQQAAFHEILHLPNLTEEQRNKFIQSLRDDPSVSLEILAEAKKLNDAQAPK

SEQ ID NO: 52 - protein, 47 aa, Artificial Sequence
  consensus sequence of variants
  Xaa (1)..(1): can be selected from I, F, Y, W, L, V
  Xaa (2)..(2): can be selected from Q or A
  Xaa (6)..(6): can be selected from D or F
  Xaa (7)..(7): can be selected from H or Y
  misc_feature (18)..(18): Xaa can be any naturally occurring amino acid
  Xaa (21)..(21): can be selected from N or H
  Xaa (22)..(22): can be selected from A or K
  Xaa (36)..(36): can be selected from E or C
  Xaa (39)..(39): can be selected from A, G, or C
  Xaa (42)..(42): can be selected from K or Q
XXQAAFXEILHLPNLTEXQRXXFIQSLRDDPSVSLXILXEAXKLNDA

SEQ ID NO: 53 - protein, 58 aa, Artificial Sequence
  cs26 N28H (203704)
IAAQHDKDQQAAFYEILHLPNLTEEQRHAFIQSLRDDPSVSLCILAEAKKLNDAQAPK

SEQ ID NO: 54 - protein, 58 aa, Artificial Sequence
  cs26 N28E (203702)
IAAQHDKDQQAAFYEILHLPNLTEEQREAFIQSLRDDPSVSLCILAEAKKLNDAQAPK

SEQ ID NO: 55 - protein, 58 aa, Artificial Sequence
  cs26 18E (204660)
IAAQHDKDQQAAFYEILELPNLTEEQRNAFIQSLRDDPSVSLCILAEAKKLNDAQAPK

SEQ ID NO: 56 - protein, 58 aa, Artificial Sequence
  cs26 L17H (203648)
IAAQHDKDQQAAFYEIHHLPNLTEEQRNAFIQSLRDDPSVSLCILAEAKKLNDAQAPK

SEQ ID NO: 57 - protein, 58 aa, Artificial Sequence
  cs26 I16H (203634)
IAAQHDKDQQAAFYEHLHLPNLTEEQRNAFIQSLRDDPSVSLCILAEAKKLNDAQAPK

SEQ ID NO: 58 - protein, 58 aa, Artificial Sequence
  cs26 Y14H (203606)
IAAQHDKDQQAAFHEILHLPNLTEEQRNAFIQSLRDDPSVSLCILAEAKKLNDAQAPK

SEQ ID NO: 59 - protein, 58 aa, Artificial Sequence
  cs26 Q10H (203564)
IAAQHDKDQHAAFYEILHLPNLTEEQRNAFIQSLRDDPSVSLCILAEAKKLNDAQAPK

SEQ ID NO: 60 - protein, 58 aa, Artificial Sequence
  cs26 Q10D (203561)
IAAQHDKDQDAAFYEILHLPNLTEEQRNAFIQSLRDDPSVSLCILAEAKKLNDAQAPK